European Patent Specification EP 3 347 470 B1, published July 9, 2025. Title: siRNA and their use in methods and compositions for inhibiting the expression of the NRARP gene. Applicant: Sylentis SAU. The sequence listing filed with the application follows.

SEQUENCE LISTING (66 sequences)

SEQ ID NO: 1 - DNA, 19 bp, Artificial Sequence
  cDNA
caccaggacatcgtgctct

SEQ ID NO: 2 - DNA, 19 bp, Artificial Sequence
  cDNA
acatcgtgctctatctcat

SEQ ID NO: 3 - DNA, 19 bp, Artificial Sequence
  cDNA
aggacatcgtgctctatct

SEQ ID NO: 4 - DNA, 19 bp, Artificial Sequence
  cDNA
gacatcgtgctctatctca

SEQ ID NO: 5 - DNA, 19 bp, Artificial Sequence
  cDNA
tgctctatctcatcaccaa

SEQ ID NO: 6 - DNA, 19 bp, Artificial Sequence
  cDNA
ccaggacatcgtgctctat

SEQ ID NO: 7 - DNA, 19 bp, Artificial Sequence
  cDNA
atcgtgctctatctcatca

SEQ ID NO: 8 - DNA, 19 bp, Artificial Sequence
  cDNA
gtgctctatctcatcacca

SEQ ID NO: 9 - DNA, 19 bp, Artificial Sequence
  cDNA
accaggacatcgtgctcta

SEQ ID NO: 10 - RNA, 19 nt, Artificial Sequence
  siRNA sense strand
caccaggacaucgugcucu

SEQ ID NO: 11 - RNA, 19 nt, Artificial Sequence
  siRNA sense strand
acaucgugcucuaucucau

SEQ ID NO: 12 - RNA, 19 nt, Artificial Sequence
  siRNA sense strand
aggacaucgugcucuaucu

SEQ ID NO: 13 - RNA, 19 nt, Artificial Sequence
  siRNA
gacaucgugcucuaucuca

SEQ ID NO: 14 - RNA, 19 nt, Artificial Sequence
  siRNA
ugcucuaucucaucaccaa

SEQ ID NO: 15 - RNA, 19 nt, Artificial Sequence
  siRNA
ccaggacaucgugcucuau

SEQ ID NO: 16 - RNA, 19 nt, Artificial Sequence
  siRNA
aucgugcucuaucucauca

SEQ ID NO: 17 - RNA, 19 nt, Artificial Sequence
  siRNA
gugcucuaucucaucacca

SEQ ID NO: 18 - RNA, 19 nt, Artificial Sequence
  siRNA
accaggacaucgugcucua

SEQ ID NO: 19 - RNA, 22 nt, Artificial Sequence
  siRNA
  modified_base 1,3,5,11,14: /mod_base="cm"
  misc_binding 4,7,20: /note="phosphothioate bond"
  modified_base 13,16,19,22: /mod_base="um"
nannnanggananngngcnncn

SEQ ID NO: 20 - RNA, 20 nt, Artificial Sequence
  siRNA
  misc_binding 2: /note="phosphothioate bond"
  modified_base 16,19: /mod_base="um"
  modified_base 18,20: /mod_base="gm"
angagcacgauguccngnnn

SEQ ID NO: 21 - RNA, 22 nt, Artificial Sequence
  siRNA
  modified_base 1,3,5,11,14: /mod_base="cm"
  misc_binding 4,7,20: /note="phosphothioate bond"
  modified_base 13,16,19,22: /mod_base="um"
nannnanggananngngcnncn

SEQ ID NO: 22 - RNA, 20 nt, Artificial Sequence
  siRNA
  misc_binding 2: /note="phosphothioate bond"
  modified_base 16,19: /mod_base="OTHER" /note="uridine with 4'-thioribose modification"
  modified_base 17,20: /mod_base="gm"
angagcacgauguccnngnn

SEQ ID NO: 23 - RNA, 22 nt, Artificial Sequence
  siRNA
  modified_base 1,3,5,11,14: /mod_base="cm"
  misc_binding 4,7,20: /note="phosphothioate bond"
  modified_base 13,16,19,22: /mod_base="um"
nannnanggananngngcnncn

SEQ ID NO: 24 - RNA, 20 nt, Artificial Sequence
  siRNA
  misc_binding 2: /note="phosphothioate bond"
  modified_base 16,19: /mod_base="OTHER" /note="5pU (5-Propynyluracile 3')"
angagcacgauguccnggng

SEQ ID NO: 25 - RNA, 22 nt, Artificial Sequence
  siRNA
  modified_base 1,3,5,11,14: /mod_base="cm"
  misc_binding 4,7,20: /note="phosphothioate bond"
  modified_base 13,16,19,22: /mod_base="um"
nannnanggananngngcnncn

SEQ ID NO: 26 - RNA, 19 nt, Artificial Sequence
  siRNA
  modified_base 15,18: /mod_base="OTHER" /note="5-methyluridine"
  modified_base 19: /mod_base="OTHER" /note="2'F Guanosine"
agagcacgauguccnggnn

SEQ ID NO: 27 - RNA, 22 nt, Artificial Sequence
  siRNA
  modified_base 1,3,5,11,14: /mod_base="cm"
  misc_binding 4,7,20: /note="phosphothioate bond"
  modified_base 13,16,19,22: /mod_base="um"
nannnanggananngngcnncn

SEQ ID NO: 28 - RNA, 19 nt, Artificial Sequence
  siRNA
  modified_base 15,18: /mod_base="um"
  modified_base 17: /mod_base="gm"
  modified_base 19: /mod_base="OTHER" /note="2'F Guanosine"
agagcacgauguccngnnn

SEQ ID NO: 29 - RNA, 22 nt, Artificial Sequence
  siRNA
  modified_base 1: /mod_base="OTHER" /note="2'F cytidine"
  modified_base 3,5,11,14: /mod_base="cm"
  misc_binding 4,7,20: /note="phosphothioate bond"
  modified_base 13,16,19,22: /mod_base="um"
nannnanggananngngcnncn

SEQ ID NO: 30 - RNA, 19 nt, Artificial Sequence
  siRNA
  modified_base 15,18: /mod_base="um"
  modified_base 17: /mod_base="gm"
  modified_base 19: /mod_base="OTHER" /note="2'F Guanosine"
agagcacgauguccngnnn

SEQ ID NO: 31 - RNA, 19 nt, Artificial Sequence
  siRNA
  modified_base 1,3,4,9,12,16,18: /mod_base="cm"
  modified_base 11,14,17,19: /mod_base="um"
nannaggananngngnnnn

SEQ ID NO: 32 - RNA, 19 nt, Artificial Sequence
  siRNA
  modified_base 1: /mod_base="OTHER" /note="2'F Adenosine"
  modified_base 5: /mod_base="cm"
  modified_base 6: /mod_base="OTHER" /note="2'-o-methyladenosine"
  modified_base 10,15,18: /mod_base="um"
ngagnncganguccnggng

SEQ ID NO: 33 - RNA, 19 nt, Artificial Sequence
  siRNA
  modified_base 1: /mod_base="OTHER" /note="2'F Cytidine"
  modified_base 3,4,9,12,16,18: /mod_base="cm"
  modified_base 11,14,17,19: /mod_base="um"
nannaggananngngnnnn

SEQ ID NO: 34 - RNA, 19 nt, Artificial Sequence
  siRNA
  modified_base 1,6: /mod_base="OTHER" /note="2'-o-methyladenosine"
  modified_base 5: /mod_base="cm"
  modified_base 10,15,18: /mod_base="um"
ngagnncganguccnggng

SEQ ID NO: 35 - RNA, 21 nt, Artificial Sequence
  siRNA
  modified_base 20,21: /mod_base="OTHER" /note="deoxithymine (2'H thymine)"
caccaggacaucgugcucunn

SEQ ID NO: 36 - RNA, 21 nt, Artificial Sequence
  siRNA
  modified_base 20,21: /mod_base="OTHER" /note="deoxithymine (2'H thymine)"
agagcacgauguccuggugnn

SEQ ID NO: 37 - RNA, 19 nt, Artificial Sequence
  siRNA
  modified_base 1,4,12,16,18: /mod_base="cm"
  modified_base 2,8,10: /mod_base="OTHER" /note="2'-o-methyladenosine"
  modified_base 3,9: /mod_base="OTHER" /note="2'F Cytidine"
  modified_base 5: /mod_base="OTHER" /note="2'F Adenosine"
  modified_base 6: /mod_base="gm"
  modified_base 7,13,15: /mod_base="OTHER" /note="2'F Guanosine"
  modified_base 11,17,19: /mod_base="OTHER" /note="2'F Uridine"
  modified_base 14: /mod_base="um"
nnnnnnnnnnnnnnnnnnn

SEQ ID NO: 38 - RNA, 19 nt, Artificial Sequence
  siRNA
  modified_base 1,6: /mod_base="OTHER" /note="2'F Adenosine"
  modified_base 2,4,8,16: /mod_base="OTHER" /note="2'F Guanosine"
  modified_base 3,9: /mod_base="OTHER" /note="2'-o-methyladenosine"
  modified_base 5,7,13: /mod_base="cm"
  modified_base 10,12,18: /mod_base="OTHER" /note="2'F Uridine"
  modified_base 11,17,19: /mod_base="gm"
  modified_base 14: /mod_base="OTHER" /note="2'F Cytidine"
  modified_base 15: /mod_base="um"
nnnnnnnnnnnnnnnnnnn

SEQ ID NO: 39 - RNA, 19 nt, Artificial Sequence
  siRNA
  modified_base 1,3,4,9,12,16,18: /mod_base="cm"
  modified_base 11,14,17,19: /mod_base="um"
nannaggananngngnnnn

SEQ ID NO: 40 - RNA, 19 nt, Artificial Sequence
  siRNA
  modified_base 5: /mod_base="cm"
agagnacgauguccuggug

SEQ ID NO: 41 - RNA, 22 nt, Artificial Sequence
  siRNA
  misc_binding 4,7,20: /note="phosphothioate bond"
  modified_base 16: /mod_base="um"
acanucngugcucuancucnau

SEQ ID NO: 42 - RNA, 19 nt, Artificial Sequence
  siRNA
  modified_base 15: /mod_base="gm"
  modified_base 17,19: /mod_base="um"
augagauagagcacnangn

SEQ ID NO: 43 - RNA, 22 nt, Artificial Sequence
  siRNA
  modified_base 2,19: /mod_base="cm"
  misc_binding 4,7,20: /note="phosphothioate bond"
  modified_base 9,14,16: /mod_base="um"
ananucngngcucnancunnau

SEQ ID NO: 44 - RNA, 19 nt, Artificial Sequence
  siRNA
  modified_base 15: /mod_base="gm"
  modified_base 17,19: /mod_base="um"
augagauagagcacnangn

SEQ ID NO: 45 - RNA, 22 nt, Artificial Sequence
  siRNA
  modified_base 2,19: /mod_base="cm"
  misc_binding 4,7,20: /note="phosphothioate bond"
  modified_base 9,14,16: /mod_base="um"
ananucngngcucnancunnau

SEQ ID NO: 46 - RNA, 19 nt, Artificial Sequence
  siRNA
  modified_base 17,19: /mod_base="OTHER" /note="5pU (5-Propynyluracile 3')"
augagauagagcacgangn

SEQ ID NO: 47 - RNA, 22 nt, Artificial Sequence
  siRNA
  modified_base 2,19: /mod_base="cm"
  misc_binding 4,7,20: /note="phosphothioate bond"
  modified_base 9,14,16: /mod_base="um"
ananucngngcucnancunnau

SEQ ID NO: 48 - RNA, 20 nt, Artificial Sequence
  siRNA
  misc_feature 2: /note="phosphothioate bond"
  modified_base 18,20: /mod_base="OTHER" /note="uridine with 4'-thioribose modification"
anugagauagagcacgangn

SEQ ID NO: 49 - RNA, 22 nt, Artificial Sequence
  siRNA
  modified_base 2,19: /mod_base="cm"
  misc_feature 4,7,20: /note="phosphothioate bond"
  modified_base 9,14,16: /mod_base="um"
ananucngngcucnancunnau

SEQ ID NO: 50 - RNA, 19 nt, Artificial Sequence
  siRNA
  modified_base 17,19: /mod_base="OTHER" /note="uridine with 4'-thioribose modification"
  modified_base 18: /mod_base="gm"
augagauagagcacgannn

SEQ ID NO: 51 - RNA, 22 nt, Artificial Sequence
  siRNA
  modified_base 2,19: /mod_base="cm"
  misc_binding 4,7,20: /note="phosphothioate bond"
  modified_base 9,14,16: /mod_base="um"
ananucngngcucnancunnau

SEQ ID NO: 52 - RNA, 19 nt, Artificial Sequence
  siRNA
  modified_base 2,17,19: /mod_base="OTHER" /note="uridine with 4'-thioribose modification"
  modified_base 18: /mod_base="gm"
angagauagagcacgannn

SEQ ID NO: 53 - RNA, 22 nt, Artificial Sequence
  siRNA
  modified_base 2,19: /mod_base="cm"
  misc_binding 4,7,20: /note="phosphothiate bond"
  modified_base 9,14,16: /mod_base="um"
ananucngngcucnancunnau

SEQ ID NO: 54 - RNA, 20 nt, Artificial Sequence
  siRNA
  misc_binding 2: /note="phosphothiate bond"
  modified_base 18,20: /mod_base="OTHER" /note="5pU (5-Propynyluracile 3')"
anugagauagagcacgangn

SEQ ID NO: 55 - RNA, 22 nt, Artificial Sequence
  siRNA
  modified_base 2,6,13,17,19: /mod_base="cm"
  misc_binding 4,7,21: /note="phosphothiate bond"
  modified_base 5,9,12,14,16,18: /mod_base="um"
anannnngngcnnnannnnanu

SEQ ID NO: 56 - RNA, 20 nt, Artificial Sequence
  siRNA
  misc_binding 2: /note="phosphothiate bond"
  modified_base 18,20: /mod_base="OTHER" /note="5'methyluridine (5mU)"
anugagauagagcacgangn

SEQ ID NO: 57 - RNA, 19 nt, Artificial Sequence
  siRNA
  modified_base 1: /mod_base="OTHER" /note="2'F Adenosine"
  modified_base 2,5,9,11,15,17: /mod_base="cm"
  modified_base 4,7,10,12,14,16,19: /mod_base="um"
nnanngngnnnnannnnan

SEQ ID NO: 58 - RNA, 19 nt, Artificial Sequence
  siRNA
  modified_base 2,7,17,19: /mod_base="um"
angaganagagcacgangn

SEQ ID NO: 59 - RNA, 19 nt, Artificial Sequence
  siRNA
  modified_base 1: /mod_base="OTHER" /note="2'-o-methyladenosine"
  modified_base 2,5,9,11,15,17: /mod_base="cm"
  modified_base 4,7,10,12,14,16,19: /mod_base="um"
nnanngngnnnnannnnan

SEQ ID NO: 60 - RNA, 19 nt, Artificial Sequence
  siRNA
  modified_base 1: /mod_base="OTHER" /note="2'F Adenosine"
  modified_base 2,7,17,19: /mod_base="um"
nngaganagagcacgangn

SEQ ID NO: 61 - RNA, 21 nt, Artificial Sequence
  siRNA
  modified_base 20,21: /mod_base="OTHER" /note="deoxithymine (2'H thymine)"
acaucgugcucuaucucaunn

SEQ ID NO: 62 - RNA, 21 nt, Artificial Sequence
  siRNA
  modified_base 20,21: /mod_base="OTHER" /note="deoxithymine (2'H thymine)"
augagauagagcacgaugunn

SEQ ID NO: 63 - RNA, 19 nt, Artificial Sequence
  siRNA
  modified_base 2,5,9,11,15,17: /mod_base="cm"
  modified_base 4,7,10,12,14,16,19: /mod_base="um"
ananngngnnnnannnnan

SEQ ID NO: 64 - RNA, 19 nt, Artificial Sequence
  siRNA
  modified_base 7: /mod_base="um"
  modified_base 12: /mod_base="cm"
augaganagagnacgaugu

SEQ ID NO: 65 - RNA, 19 nt, Artificial Sequence
  siRNA
  modified_base 1,18: /mod_base="OTHER" /note="2'-o-methyladenosine"
  modified_base 2: /mod_base="cm"
  modified_base 3,13: /mod_base="OTHER" /note="2'F Adenosine"
  modified_base 4,10,12,14,16: /mod_base="um"
  modified_base 5,9,11,15,17: /mod_base="OTHER" /note="2'F Cytidine"
  modified_base 6,8: /mod_base="gm"
  modified_base 7,19: /mod_base="OTHER" /note="2'F Uridine"
nnnnnnnnnnnnnnnnnnn

SEQ ID NO: 66 - RNA, 19 nt, Artificial Sequence
  siRNA
  modified_base 1,4,6,8,10,16: /mod_base="OTHER" /note="2'F Adenosine"
  modified_base 2: /mod_base="OTHER" /note="2'F Uridine"
  modified_base 3,5,9,11,15: /mod_base="gm"
  modified_base 7,17,19: /mod_base="um"
  modified_base 12: /mod_base="OTHER" /note="2'F Cytidine"
  modified_base 18: /mod_base="OTHER" /note="2'F Guanosine"
nnnnnnnnnnnnacnnnnn